European Patent Application EP 4 814 019 A1, published September 30, 2026. Title: 一种抗NY-ESO-1的纳米抗体及其应用. Applicant: 浙江大学. The sequence listing filed with the application follows.

SEQUENCE LISTING (46 sequences)

SEQ ID NO: 1 - protein, 9 aa, synthetic construct
GTIFHQIDM

SEQ ID NO: 2 - protein, 14 aa, synthetic construct
ELVAAIGTGSSTYY

SEQ ID NO: 3 - protein, 11 aa, synthetic construct
AVYYCAAWHYY

SEQ ID NO: 4 - protein, 112 aa, synthetic construct
QVQLQESGGGLVQAGGSLRLSCAASGTIFHQIDMGWYRQAPGKERELVAAIGTGSSTYYADSVKGRFTISRDNAKNTVYLQMNSLKPEDTAVYYCAAWHYYWGQGTQVTVSS

SEQ ID NO: 5 - DNA, 336 bp, synthetic construct
  source 1..336: mol_type = other DNA
caggtgcagctgcaggaaagcggcggcggcctggtgcaggcgggcggcagcctgcgcctgagctgcgcggcgagcggcactatttttcatcagatcgacatgggctggtatcgccaggcgccgggcaaagaacgcgaacttgttgccgctattggtactggtagtagtacctattatgcggatagcgtgaaaggccgctttaccattagccgcgataacgcgaaaaacaccgtgtatctgcagatgaacagcctgaaaccggaagataccgcggtgtattattgcgcggcttggcattactattggggccagggcacccaggtgaccgtgagcagc

SEQ ID NO: 6 - protein, 9 aa, synthetic construct
GNIFYPQYM

SEQ ID NO: 7 - protein, 14 aa, synthetic construct
EFVAAISDGASTYY

SEQ ID NO: 8 - protein, 10 aa, synthetic construct
AVYYCADLWY

SEQ ID NO: 9 - protein, 111 aa, synthetic construct
QVQLQESGGGLVQAGGSLRLSCAASGNIFYPQYMGWYRQAPGKEREFVAAISDGASTYYADSVKGRFTISRDNAKNTVYLQMNSLKPEDTAVYYCADLWYWGQGTQVTVSS

SEQ ID NO: 10 - DNA, 333 bp, synthetic construct
  source 1..333: mol_type = other DNA
caggtgcagctgcaggaaagcggcggcggcctggtgcaggcgggcggcagcctgcgcctgagctgcgcggcgagcggcaatattttttacccgcagtacatgggctggtatcgccaggcgccgggcaaagaacgcgaatttgttgccgctattagtgacggtgctagtacctattatgcggatagcgtgaaaggccgctttaccattagccgcgataacgcgaaaaacaccgtgtatctgcagatgaacagcctgaaaccggaagataccgcggtgtattattgcgcggacctttggtattggggccagggcacccaggtgaccgtgagcagc

SEQ ID NO: 11 - protein, 9 aa, synthetic construct
GNISAVYTM

SEQ ID NO: 12 - protein, 14 aa, synthetic construct
EFVAAIDYGGSTYY

SEQ ID NO: 13 - protein, 12 aa, synthetic construct
AVYYCASYYHGY

SEQ ID NO: 14 - protein, 113 aa, synthetic construct
QVQLQESGGGLVQAGGSLRLSCAASGNISAVYTMGWYRQAPGKEREFVAAIDYGGSTYYADSVKGRFTISRDNAKNTVYLQMNSLKPEDTAVYYCASYYHGYWGQGTQVTVSS

SEQ ID NO: 15 - DNA, 339 bp, synthetic construct
  source 1..339: mol_type = other DNA
caggtgcagctgcaggaaagcggcggcggcctggtgcaggcgggcggcagcctgcgcctgagctgcgcggcgagcggcaatatttctgctgtttacactatgggctggtatcgccaggcgccgggcaaagaacgcgaatttgttgccgctattgattacggtggtagtacctattatgcggatagcgtgaaaggccgctttaccattagccgcgataacgcgaaaaacaccgtgtatctgcagatgaacagcctgaaaccggaagataccgcggtgtattattgcgcgtcttactaccatggttattggggccagggcacccaggtgaccgtgagcagc

SEQ ID NO: 16 - protein, 9 aa, synthetic construct
GYISYLNTM

SEQ ID NO: 17 - protein, 14 aa, synthetic construct
EFVATIGQGSSTYY

SEQ ID NO: 18 - protein, 11 aa, synthetic construct
AVYYCADQLGY

SEQ ID NO: 19 - protein, 112 aa, synthetic construct
QVQLQESGGGLVQAGGSLRLSCAASGYISYLNTMGWYRQAPGKEREFVATIGQGSSTYYADSVKGRFTISRDNAKNTVYLQMNSLKPEDTAVYYCADQLGYWGQGTQVTVSS

SEQ ID NO: 20 - DNA, 336 bp, synthetic construct
  source 1..336: mol_type = other DNA
caggtgcagctgcaggaaagcggcggcggcctggtgcaggcgggcggcagcctgcgcctgagctgcgcggcgagcggctatatttcttacctgaacactatgggctggtatcgccaggcgccgggcaaagaacgcgaatttgttgccactattggtcagggtagtagtacctattatgcggatagcgtgaaaggccgctttaccattagccgcgataacgcgaaaaacaccgtgtatctgcagatgaacagcctgaaaccggaagataccgcggtgtattattgcgcggaccagcttggttattggggccagggcacccaggtgaccgtgagcagc

SEQ ID NO: 21 - protein, 349 aa, synthetic construct
QVQLQESGGGLVQAGGSLRLSCAASGNISAVYTMGWYRQAPGKEREFVAAIDYGGSTYYADSVKGRFTISRDNAKNTVYLQMNSLKPEDTAVYYCASYYHGYWGQGTQVTVSSGGGGSPKSCDKTHTCPPCPAPELLGGPSVFLFPPKPKDTLMISRTPEVTCVVVDVSHEDPEVKFNWYVDGVEVHNAKTKPREEQYNSTYRVVSVLTVLHQDWLNGKEYKCKVSNKALPAPIEKTISKAKGQPREPQVYTLPPSREEMTKNQVSLTCLVKGFYPSDIAVEWESNGQPENNYKTTPPVLDSDGSFFLYSKLTVDKSRWQQGNVFSCSVMHEALHNHYTQKSLSLSPGK

SEQ ID NO: 22 - DNA, 1047 bp, synthetic construct
  source 1..1047: mol_type = other DNA
caggtgcagctgcaggagagcggcggcggcctggtgcaggccggcggcagcctgagactgtcttgtgccgcctctggcaatattagcgccgtgtatacaatgggctggtatagacaggcccctggcaaagagagagagttcgtggccgccattgattatggcggcagcacatattatgccgatagcgtgaaaggcagattcacaatttctagagataatgccaaaaatacagtgtatctgcagatgaatagcctgaaacctgaggatacagccgtgtattattgtgcctcttattatcatggctattggggccagggcacacaggtgacagtgtctagcggaggtggtggctctcccaaatcttgtgacaaaactcacacatgcccaccgtgcccagcacctgaactcctggggggaccgtcagtcttcctcttccccccaaaacccaaggacaccctcatgatctcccggacccctgaggtcacatgcgtggtggtggacgtgagccacgaagaccctgaggtcaagttcaactggtacgtggacggcgtggaggtgcataatgccaagacaaagccgcgggaggagcagtacaacagcacgtaccgtgtggtcagcgtcctcaccgtcctgcaccaggactggctgaatggcaaggagtacaagtgcaaggtctccaacaaagccctcccagcccccatcgagaaaaccatctccaaagccaaagggcagccccgagaaccacaggtgtacaccctgcccccatcccgggaggagatgaccaagaaccaggtcagcctgacctgcctggtcaaaggcttctatcccagcgacatcgccgtggagtgggagagcaatgggcagccggagaacaactacaagaccacgcctcccgtgctggactccgacggctccttcttcctctacagcaagctcaccgtggacaagagcaggtggcagcaggggaacgtcttctcatgctccgtgatgcatgaggctctgcacaaccactacacgcagaagagcctctccctgtctccgggtaaa

SEQ ID NO: 23 - protein, 458 aa, synthetic construct
QVQLQESGGGLVQAGGSLRLSCAASGNISAVYTMGWYRQAPGKEREFVAAIDYGGSTYYADSVKGRFTISRDNAKNTVYLQMNSLKPEDTAVYYCASYYHGYWGQGTQVTVSSGGGGSGGGGSGGGGSASTKGPSVFPLAPSSKSTSGGTAALGCLVKDYFPEPVTVSWNSGALTSGVHTFPAVLQSSGLYSLSSVVTVPSSSLGTQTYICNVNHKPSNTKVDKKVEPKSCDKTHTCPPCPAPEAAGGPSVFLFPPKPKDTLMISRTPEVTCVVVDVSHEDPEVKFNWYVDGVEVHNAKTKPREEQYNSTYRVVSVLTVLHQDWLNGKEYKCKVSNKALGAPIEKTISKAKGQPREPQVYTLPPSREEMTKNQVSLTCLVKGFYPSDIAVEWESNGQPENNYKTTPPVLDSDGSFFLYSKLTVDKSRWQQGNVFSCSVMHEALHNHYTQKSLSLSPGK

SEQ ID NO: 24 - DNA, 1374 bp, synthetic construct
  source 1..1374: mol_type = other DNA
caggtgcagctgcaggagagcggcggcggcctggtgcaggccggcggcagcctgagactgtcttgtgccgcctctggcaatattagcgccgtgtatacaatgggctggtatagacaggcccctggcaaagagagagagttcgtggccgccattgattatggcggcagcacatattatgccgatagcgtgaaaggcagattcacaatttctagagataatgccaaaaatacagtgtatctgcagatgaatagcctgaaacctgaggatacagccgtgtattattgtgcctcttattatcatggctattggggccagggcacacaggtgacagtgtctagcggaggaggcggctctggaggaggcggctctggaggaggcggctctgctagcaccaagggcccatcggtcttccccctggcaccctcctccaagagcacctctgggggcacagcggccctgggctgcctggtcaaggactacttccccgaaccggtgacggtgtcgtggaactcaggcgccctgaccagcggcgtgcacaccttcccggctgtcctacagtcctcaggactctactccctcagcagcgtggtgaccgtgccctccagcagcttgggcacccagacctacatctgcaacgtgaatcacaagcccagcaacaccaaggtggacaagaaagttgagcccaaatcttgtgacaaaactcacacatgcccaccgtgcccagcacctgaagccgctgggggaccgtcagtcttcctcttccccccaaaacccaaggacaccctcatgatctcccggacccctgaggtcacatgcgtggtggtggacgtgagccacgaagaccctgaggtcaagttcaactggtacgtggacggcgtggaggtgcataatgccaagacaaagccgcgggaggagcagtacaacagcacgtaccgtgtggtcagcgtcctcaccgtcctgcaccaggactggctgaatggcaaggagtacaagtgcaaggtctccaacaaagccctcggagcccccatcgagaaaaccatctccaaagccaaagggcagccccgagaaccacaggtgtacaccctgcccccatcccgggaggagatgaccaagaaccaggtcagcctgacctgcctggtcaaaggcttctatcccagcgacatcgccgtggagtgggagagcaatgggcagccggagaacaactacaagaccacgcctcccgtgctggactccgacggctccttcttcctctacagcaagctcaccgtggacaagagcaggtggcagcaggggaacgtcttctcatgctccgtgatgcatgaggctctgcacaaccactacacgcagaagagcctctccctgtctccgggtaaa

SEQ ID NO: 25 - protein, 235 aa, synthetic construct
QVQLQESGGGLVQAGGSLRLSCAASGNISAVYTMGWYRQAPGKEREFVAAIDYGGSTYYADSVKGRFTISRDNAKNTVYLQMNSLKPEDTAVYYCASYYHGYWGQGTQVTVSSGGGGSGGGGSGGGGSRTVAAPSVFIFPPSDEQLKSGTASVVCLLNNFYPREAKVQWKVDNALQSGNSQESVTEQDSKDSTYSLSSTLTLSKADYEKHKVYACEVTHQGLSSPVTKSFNRGEC

SEQ ID NO: 26 - DNA, 705 bp, synthetic construct
  source 1..705: mol_type = other DNA
caggtgcagctgcaggagagcggcggcggcctggtgcaggccggcggcagcctgagactgtcttgtgccgcctctggcaatattagcgccgtgtatacaatgggctggtatagacaggcccctggcaaagagagagagttcgtggccgccattgattatggcggcagcacatattatgccgatagcgtgaaaggcagattcacaatttctagagataatgccaaaaatacagtgtatctgcagatgaatagcctgaaacctgaggatacagccgtgtattattgtgcctcttattatcatggctattggggccagggcacacaggtgacagtgtctagcggaggaggcggctctggaggaggcggctctggaggaggcggctctcgtacggtggctgcaccatctgtcttcatcttcccgccatctgatgagcagttgaaatctggaactgcctctgttgtgtgcctgctgaataacttctatcccagagaggccaaagtacagtggaaggtggataacgccctccaatcgggtaactcccaggagagtgtcacagagcaggacagcaaggacagcacctacagcctcagcagcaccctgacgctgagcaaagcagactacgagaaacacaaagtctacgcctgcgaagtcacccatcagggcctgagctcgcccgtcacaaagagcttcaacaggggagagtgt

SEQ ID NO: 27 - protein, 9 aa, synthetic construct
SLLMWITQC

SEQ ID NO: 28 - DNA, 50 bp, synthetic construct
  source 1..50: mol_type = other DNA
caggtgcagctgcaggaaagcggcggcggcctggtgcaggcgggcggcag

SEQ ID NO: 29 - DNA, 43 bp, synthetic construct
  source 1..43: mol_type = other DNA
gccgctcgccgcgcagctcaggcgcaggctgccgcccgcctgc

SEQ ID NO: 30 - DNA, 45 bp, synthetic construct
  source 1..45: mol_type = other DNA
cgcggcgagcggcwmtatttytnnnnatgggctggtatcgccagg

SEQ ID NO: 31 - DNA, 39 bp, synthetic construct
  source 1..39: mol_type = other DNA
ttcgcgttctttgcccggcgcctggcgataccagcccat

SEQ ID NO: 32 - DNA, 74 bp, synthetic construct
  source 1..74: mol_type = other DNA
ccgggcaaagaacgcgaayttgttgccrstattrvtnggtrstantaccwattatgcggatagcgtgaaaggcc

SEQ ID NO: 33 - DNA, 54 bp, synthetic construct
  source 1..54: mol_type = other DNA
gtttttcgcgttatcgcggctaatggtaaagcggcctttcacgctatccgcata

SEQ ID NO: 34 - DNA, 53 bp, synthetic construct
  source 1..53: mol_type = other DNA
agccgcgataacgcgaaaaacaccgtgtatctgcagatgaacagcctgaaacc

SEQ ID NO: 35 - DNA, 52 bp, synthetic construct
  source 1..52: mol_type = other DNA
cgcgcaataatacaccgcggtatcttccggtttcaggctgttcatctgcaga

SEQ ID NO: 36 - DNA, 52 bp, synthetic construct
  source 1..52: mol_type = other DNA
ccgcggtgtattattgcgcggytnnnnnnnywtntattggggccagggcacc

SEQ ID NO: 37 - DNA, 56 bp, synthetic construct
  source 1..56: mol_type = other DNA
ccgcggtgtattattgcgcggytnnnnnnnnnnnywtntattggggccagggcacc

SEQ ID NO: 38 - DNA, 60 bp, synthetic construct
  source 1..60: mol_type = other DNA
ccgcggtgtattattgcgcggytnnnnnnnnnnnnnnnywtntattggggccagggcacc

SEQ ID NO: 39 - DNA, 36 bp, synthetic construct
  source 1..36: mol_type = other DNA
gctgctcacggtcacctgggtgccctggccccaata

SEQ ID NO: 40 - DNA, 47 bp, synthetic construct
  source 1..47: mol_type = other DNA
ctcctcgctgcccagccggcgatggcccaggtgcagctgcaggaaag

SEQ ID NO: 41 - DNA, 46 bp, synthetic construct
  source 1..46: mol_type = other DNA
cggatctcagtggtggtggtggtggtggctgctcacggtcacctgg

SEQ ID NO: 42 - DNA, 60 bp, synthetic construct
  source 1..60: mol_type = other DNA
gaaggtgttcaattggacaagagagaagctgacgcacaggtgcagctgcaggaaagcggc

SEQ ID NO: 43 - DNA, 90 bp, synthetic construct
  source 1..90: mol_type = other DNA
tactgatgcttctgtagagggtgaggatgtttgagcgtaatctggaacatcgtatgggtaggatccgctgctcacggtcacctgggtgcc

SEQ ID NO: 44 - DNA, 59 bp, synthetic construct
  source 1..59: mol_type = other DNA
accaccatcgcttctatcgctgctaaggaagaaggtgttcaattggacaagagagaagc

SEQ ID NO: 45 - DNA, 26 bp, synthetic construct
  source 1..26: mol_type = other DNA
tactgatgcttctgtagagggtgagg

SEQ ID NO: 46 - DNA, 27 bp, synthetic construct
  source 1..27: mol_type = other DNA
accaccatcgcttctatcgctgctaag